European Patent Application EP 4 534 656 A1, published April 9, 2025. Title: DNA methyltransferase. Applicant: 国立大学法人九州大学. The sequence listing filed with the application follows.

SEQUENCE LISTING (10 sequences)

SEQ ID NO: 1 - DNA, 1089 bp, Paramecium bursaria Chlorella virus NY2A
  source 1..1089: mol_type = genomic DNA
  CDS 1..1089: protein_id = 2; translation = MRTKYRIFIVCMLMSMKALELFAGIGGITHGLRGYVEPIAFCEYEKDASSFLSQRGLPVHGDITKFDASVYKNKIDIVTAGWPCTGFSTAGKGTGFEHEASGLWTEVVRVVKESEPKYVFLENSHVLAQTKNLKVIIHDLDNLGYDTRWWTCRSNDVNVGAHHNRYRWFMLAEKKGSVTKFVKIQVKKFNWSGDFKEKQISENSHENKQLIKFMGNSVVPDQVRYAFESMSDMILEGSLVNEKDEIVKVGYSKDSIMYKIPIEHKIIPKLNIVLTPRDPPEGHKAREEAIIKSPILMTYWNTPAFCYHKSARGAKILTKRQKNNLHTQIKFCPGGSDDGYLSGRFCAWLMGYDDEYLGDLMHY
atgcgcacgaaataccgcatcttcatcgtctgcatgctgatgtccatgaaagccttggaactatttgcggggataggtggcattacccatggcttacgtggctatgtagaaccgattgcattctgcgaatatgagaaagatgccagctcgtttctgtcacaacgtggcttacccgttcatggggacattacgaagtttgacgccagtgtgtacaaaaacaagattgacattgtgacagcaggatggccttgtactgggttttcgaccgcgggtaaaggcactggttttgagcatgaagctagcggtttatggacagaagtggtccgagtagtgaaagagagcgaaccgaaatacgtctttttggaaaatagtcacgttttggcgcaaaccaaaaacctcaaggtcatcatccatgatctggataaccttggctatgatacgcgttggtggacgtgcagatcgaatgacgttaatgtcggtgcacatcacaatcggtatcgctggtttatgctcgcagagaaaaaaggctctgtgaccaaattcgtgaaaattcaggtgaaaaagttcaattggtctggtgacttcaaagagaaacagataagcgagaacagtcacgaaaacaagcagctcattaagttcatgggaaactccgtagttccggatcaagttcgctatgcgtttgaatcgatgagcgacatgattctggaaggcagtctggtgaatgaaaaggatgagatcgtgaaggtaggctattccaaagatagcatcatgtacaaaattccgattgaacacaaaatcattccgaaacttaacatcgttctgaccccacgtgatccgccagaaggccataaagcccgtgaagaagcgatcatcaaaagccccattctgatgacgtactggaatactccggccttttgctatcacaaatcagctcgcggcgctaaaattctgaccaaacgtcagaaaaacaacctgcatacccagatcaaattctgtcctggtggttctgacgatggttatctgtcaggtcgcttttgtgcgtggctgatgggatacgatgatgaatacctgggggatcttatgcactat

SEQ ID NO: 2 - protein, 363 aa, Paramecium bursaria Chlorella virus NY2A
MRTKYRIFIVCMLMSMKALELFAGIGGITHGLRGYVEPIAFCEYEKDASSFLSQRGLPVHGDITKFDASVYKNKIDIVTAGWPCTGFSTAGKGTGFEHEASGLWTEVVRVVKESEPKYVFLENSHVLAQTKNLKVIIHDLDNLGYDTRWWTCRSNDVNVGAHHNRYRWFMLAEKKGSVTKFVKIQVKKFNWSGDFKEKQISENSHENKQLIKFMGNSVVPDQVRYAFESMSDMILEGSLVNEKDEIVKVGYSKDSIMYKIPIEHKIIPKLNIVLTPRDPPEGHKAREEAIIKSPILMTYWNTPAFCYHKSARGAKILTKRQKNNLHTQIKFCPGGSDDGYLSGRFCAWLMGYDDEYLGDLMHY

SEQ ID NO: 3 - DNA, 1089 bp, Chlorella virus
  source 1..1089: mol_type = genomic DNA
  CDS 1..1089: protein_id = 4; translation = MRTKYRIFIVCMLMSMKALELFAGIGGITHGLRGYVEPIAFCEYEKDASSFLSQRGLPVHGDITKFDASVYKNKIDIVTAGWPCTGFSTAGKGTGFEHEASGLWTEVVRVVKESEPKYVFLENSHVLAQTKNLKVIIHDLDILGYDTRWWTCRSNDVNVGAHHNRYRWFMLAEKKGSVTKFVKIQVKKFNWSGDFKEKQISENSHENKQLIKFMGNSVVPDQVRYAFESMSDMILEGSLVNDKDEIVKVGYSKDGIMYKIPIEHKIIPKLNIVLTPRDPPEGHKAREEAIIKSPILMTYWNTPAFCYHKSARGAKILTKRQKNNLHTQIKFCPGGSDDGYLSGRFCAWLMGYDDEYLGDLMHY
atgcgcacgaaataccgcatcttcatcgtctgcatgctgatgtccatgaaagccttggaactatttgcggggataggtggcattacccatggcttacgtggctatgtagaaccgattgcattctgcgaatatgagaaagatgccagctcgtttctgtcacaacgtggcttacccgttcatggggacattacgaagtttgacgccagtgtgtacaaaaacaagattgacattgtgacagcaggatggccttgtactgggttttcgaccgcgggtaaaggcactggttttgagcatgaagctagcggtttatggacagaagtggtccgagtagtgaaagagagcgaaccgaaatacgtctttttggaaaatagtcacgttttggcgcaaaccaaaaacctcaaggtcatcatccatgatctggatatccttggctatgatacgcgttggtggacgtgcagatcgaatgacgttaatgtcggtgcacatcacaatcggtatcgctggtttatgctcgcagagaaaaaaggctctgtgaccaaattcgtgaaaattcaggtgaaaaagttcaattggtctggtgacttcaaagagaaacagataagcgagaacagtcacgaaaacaagcagctcattaagttcatgggaaactccgtagttccggatcaagttcgctatgcgtttgaatcgatgagcgacatgattctggaaggcagtctggtgaatgataaggatgagatcgtgaaggtaggctattccaaagatggcatcatgtacaaaattccgattgaacacaaaatcattccgaaacttaacatcgttctgaccccacgtgatccgccagaaggccataaagcccgtgaagaagcgatcatcaaaagccccattctgatgacgtactggaatactccggccttttgctatcacaaatcagctcgcggcgctaaaattctgaccaaacgtcagaaaaacaacctgcatacccagatcaaattctgtcctggtggttctgacgatggttatctgtcaggtcgcttttgtgcgtggctgatgggatacgatgatgaatacctgggggatcttatgcactat

SEQ ID NO: 4 - protein, 363 aa, Chlorella virus
MRTKYRIFIVCMLMSMKALELFAGIGGITHGLRGYVEPIAFCEYEKDASSFLSQRGLPVHGDITKFDASVYKNKIDIVTAGWPCTGFSTAGKGTGFEHEASGLWTEVVRVVKESEPKYVFLENSHVLAQTKNLKVIIHDLDILGYDTRWWTCRSNDVNVGAHHNRYRWFMLAEKKGSVTKFVKIQVKKFNWSGDFKEKQISENSHENKQLIKFMGNSVVPDQVRYAFESMSDMILEGSLVNDKDEIVKVGYSKDGIMYKIPIEHKIIPKLNIVLTPRDPPEGHKAREEAIIKSPILMTYWNTPAFCYHKSARGAKILTKRQKNNLHTQIKFCPGGSDDGYLSGRFCAWLMGYDDEYLGDLMHY

SEQ ID NO: 5 - DNA, 1044 bp, synthetic construct
  misc_feature 1..1044: note = Recombinant DNA
  source 1..1044: mol_type = other DNA
  CDS 1..1044: protein_id = 6; translation = MKALELFAGIGGITHGLRGYVEPIAFCEYEKDASSFLSQRGLPVHGDITKFDASVYKNKIDIVTAGWPCTGFSTAGKGTGFEHEASGLWTEVVRVVKESEPKYVFLENSHVLAQTKNLKVIIHDLDNLGYDTRWWTCRSNDVNVGAHHNRYRWFMLAEKKGSVTKFVKIQVKKFNWSGDFKEKQISENSHENKQLIKFMGNSVVPDQVRYAFESMSDMILEGSLVNEKDEIVKVGYSKDSIMYKIPIEHKIIPKLNIVLTPRDPPEGHKAREEAIIKSPILMTYWNTPAFCYHKSARGAKILTKRQKNNLHTQIKFCPGGSDDGYLSGRFCAWLMGYDDEYLGDLMHY
atgaaagccttggaactatttgcggggataggtggcattacccatggcttacgtggctatgtagaaccgattgcattctgcgaatatgagaaagatgccagctcgtttctgtcacaacgtggcttacccgttcatggggacattacgaagtttgacgccagtgtgtacaaaaacaagattgacattgtgacagcaggatggccttgtactgggttttcgaccgcgggtaaaggcactggttttgagcatgaagctagcggtttatggacagaagtggtccgagtagtgaaagagagcgaaccgaaatacgtctttttggaaaatagtcacgttttggcgcaaaccaaaaacctcaaggtcatcatccatgatctggataaccttggctatgatacgcgttggtggacgtgcagatcgaatgacgttaatgtcggtgcacatcacaatcggtatcgctggtttatgctcgcagagaaaaaaggctctgtgaccaaattcgtgaaaattcaggtgaaaaagttcaattggtctggtgacttcaaagagaaacagataagcgagaacagtcacgaaaacaagcagctcattaagttcatgggaaactccgtagttccggatcaagttcgctatgcgtttgaatcgatgagcgacatgattctggaaggcagtctggtgaatgaaaaggatgagatcgtgaaggtaggctattccaaagatagcatcatgtacaaaattccgattgaacacaaaatcattccgaaacttaacatcgttctgaccccacgtgatccgccagaaggccataaagcccgtgaagaagcgatcatcaaaagccccattctgatgacgtactggaatactccggccttttgctatcacaaatcagctcgcggcgctaaaattctgaccaaacgtcagaaaaacaacctgcatacccagatcaaattctgtcctggtggttctgacgatggttatctgtcaggtcgcttttgtgcgtggctgatgggatacgatgatgaatacctgggggatcttatgcactat

SEQ ID NO: 6 - protein, 348 aa, synthetic construct
  REGION 1..348: note = Recombinant Protein
MKALELFAGIGGITHGLRGYVEPIAFCEYEKDASSFLSQRGLPVHGDITKFDASVYKNKIDIVTAGWPCTGFSTAGKGTGFEHEASGLWTEVVRVVKESEPKYVFLENSHVLAQTKNLKVIIHDLDNLGYDTRWWTCRSNDVNVGAHHNRYRWFMLAEKKGSVTKFVKIQVKKFNWSGDFKEKQISENSHENKQLIKFMGNSVVPDQVRYAFESMSDMILEGSLVNEKDEIVKVGYSKDSIMYKIPIEHKIIPKLNIVLTPRDPPEGHKAREEAIIKSPILMTYWNTPAFCYHKSARGAKILTKRQKNNLHTQIKFCPGGSDDGYLSGRFCAWLMGYDDEYLGDLMHY

SEQ ID NO: 7 - DNA, 1044 bp, synthetic construct
  misc_feature 1..1044: note = Recombinant DNA
  source 1..1044: mol_type = other DNA
  CDS 1..1044: protein_id = 8; translation = MKALELFAGIGGITHGLRGYVEPIAFCEYEKDASSFLSQRGLPVHGDITKFDASVYKNKIDIVTAGWPCTGFSTAGKGTGFEHEASGLWTEVVRVVKESEPKYVFLENSHVLAQTKNLKVIIHDLDILGYDTRWWTCRSNDVNVGAHHNRYRWFMLAEKKGSVTKFVKIQVKKFNWSGDFKEKQISENSHENKQLIKFMGNSVVPDQVRYAFESMSDMILEGSLVNDKDEIVKVGYSKDGIMYKIPIEHKIIPKLNIVLTPRDPPEGHKAREEAIIKSPILMTYWNTPAFCYHKSARGAKILTKRQKNNLHTQIKFCPGGSDDGYLSGRFCAWLMGYDDEYLGDLMHY
atgaaagccttggaactatttgcggggataggtggcattacccatggcttacgtggctatgtagaaccgattgcattctgcgaatatgagaaagatgccagctcgtttctgtcacaacgtggcttacccgttcatggggacattacgaagtttgacgccagtgtgtacaaaaacaagattgacattgtgacagcaggatggccttgtactgggttttcgaccgcgggtaaaggcactggttttgagcatgaagctagcggtttatggacagaagtggtccgagtagtgaaagagagcgaaccgaaatacgtctttttggaaaatagtcacgttttggcgcaaaccaaaaacctcaaggtcatcatccatgatctggatatccttggctatgatacgcgttggtggacgtgcagatcgaatgacgttaatgtcggtgcacatcacaatcggtatcgctggtttatgctcgcagagaaaaaaggctctgtgaccaaattcgtgaaaattcaggtgaaaaagttcaattggtctggtgacttcaaagagaaacagataagcgagaacagtcacgaaaacaagcagctcattaagttcatgggaaactccgtagttccggatcaagttcgctatgcgtttgaatcgatgagcgacatgattctggaaggcagtctggtgaatgataaggatgagatcgtgaaggtaggctattccaaagatggcatcatgtacaaaattccgattgaacacaaaatcattccgaaacttaacatcgttctgaccccacgtgatccgccagaaggccataaagcccgtgaagaagcgatcatcaaaagccccattctgatgacgtactggaatactccggccttttgctatcacaaatcagctcgcggcgctaaaattctgaccaaacgtcagaaaaacaacctgcatacccagatcaaattctgtcctggtggttctgacgatggttatctgtcaggtcgcttttgtgcgtggctgatgggatacgatgatgaatacctgggggatcttatgcactat

SEQ ID NO: 8 - protein, 348 aa, synthetic construct
  REGION 1..348: note = Recombinant Protein
MKALELFAGIGGITHGLRGYVEPIAFCEYEKDASSFLSQRGLPVHGDITKFDASVYKNKIDIVTAGWPCTGFSTAGKGTGFEHEASGLWTEVVRVVKESEPKYVFLENSHVLAQTKNLKVIIHDLDILGYDTRWWTCRSNDVNVGAHHNRYRWFMLAEKKGSVTKFVKIQVKKFNWSGDFKEKQISENSHENKQLIKFMGNSVVPDQVRYAFESMSDMILEGSLVNDKDEIVKVGYSKDGIMYKIPIEHKIIPKLNIVLTPRDPPEGHKAREEAIIKSPILMTYWNTPAFCYHKSARGAKILTKRQKNNLHTQIKFCPGGSDDGYLSGRFCAWLMGYDDEYLGDLMHY

SEQ ID NO: 9 - DNA, 1101 bp, synthetic construct
  misc_feature 1..1101: note = Synthetic DNA
  source 1..1101: mol_type = other DNA
ggatccatgcgcacgaaataccgcatcttcatcgtctgcatgctgatgtccatgaaagccttggaactatttgcggggataggtggcattacccatggcttacgtggctatgtagaaccgattgcattctgcgaatatgagaaagatgccagctcgtttctgtcacaacgtggcttacccgttcatggggacattacgaagtttgacgccagtgtgtacaaaaacaagattgacattgtgacagcaggatggccttgtactgggttttcgaccgcgggtaaaggcactggttttgagcatgaagctagcggtttatggacagaagtggtccgagtagtgaaagagagcgaaccgaaatacgtctttttggaaaatagtcacgttttggcgcaaaccaaaaacctcaaggtcatcatccatgatctggataaccttggctatgatacgcgttggtggacgtgcagatcgaatgacgttaatgtcggtgcacatcacaatcggtatcgctggtttatgctcgcagagaaaaaaggctctgtgaccaaattcgtgaaaattcaggtgaaaaagttcaattggtctggtgacttcaaagagaaacagataagcgagaacagtcacgaaaacaagcagctcattaagttcatgggaaactccgtagttccggatcaagttcgctatgcgtttgaatcgatgagcgacatgattctggaaggcagtctggtgaatgaaaaggatgagatcgtgaaggtaggctattccaaagatagcatcatgtacaaaattccgattgaacacaaaatcattccgaaacttaacatcgttctgaccccacgtgatccgccagaaggccataaagcccgtgaagaagcgatcatcaaaagccccattctgatgacgtactggaatactccggccttttgctatcacaaatcagctcgcggcgctaaaattctgaccaaacgtcagaaaaacaacctgcatacccagatcaaattctgtcctggtggttctgacgatggttatctgtcaggtcgcttttgtgcgtggctgatgggatacgatgatgaatacctgggggatcttatgcactatgaattc

SEQ ID NO: 10 - DNA, 1110 bp, synthetic construct
  misc_feature 1..1110: note = Synthetic DNA
  source 1..1110: mol_type = other DNA
atgaaagccggatccatgcgcacgaaataccgcatcttcatcgtctgcatgctgatgtccatgaaagccttggaactatttgcggggataggtggcattacccatggcttacgtggctatgtagaaccgattgcattctgcgaatatgagaaagatgccagctcgtttctgtcacaacgtggcttacccgttcatggggacattacgaagtttgacgccagtgtgtacaaaaacaagattgacattgtgacagcaggatggccttgtactgggttttcgaccgcgggtaaaggcactggttttgagcatgaagctagcggtttatggacagaagtggtccgagtagtgaaagagagcgaaccgaaatacgtctttttggaaaatagtcacgttttggcgcaaaccaaaaacctcaaggtcatcatccatgatctggatatccttggctatgatacgcgttggtggacgtgcagatcgaatgacgttaatgtcggtgcacatcacaatcggtatcgctggtttatgctcgcagagaaaaaaggctctgtgaccaaattcgtgaaaattcaggtgaaaaagttcaattggtctggtgacttcaaagagaaacagataagcgagaacagtcacgaaaacaagcagctcattaagttcatgggaaactccgtagttccggatcaagttcgctatgcgtttgaatcgatgagcgacatgattctggaaggcagtctggtgaatgataaggatgagatcgtgaaggtaggctattccaaagatggcatcatgtacaaaattccgattgaacacaaaatcattccgaaacttaacatcgttctgaccccacgtgatccgccagaaggccataaagcccgtgaagaagcgatcatcaaaagccccattctgatgacgtactggaatactccggccttttgctatcacaaatcagctcgcggcgctaaaattctgaccaaacgtcagaaaaacaacctgcatacccagatcaaattctgtcctggtggttctgacgatggttatctgtcaggtcgcttttgtgcgtggctgatgggatacgatgatgaatacctgggggatcttatgcactatgaattc